European Patent Specification EP 3 741 283 B1, published March 19, 2025. Title: AUTOMATIC DISHWASHING METHOD. Applicant: Procter & Gamble. The sequence listing filed with the application follows.

SEQUENCE LISTING (6 sequences)

SEQ ID NO: 1 - protein, 237 aa, Bacillus agaradhaerens
MLTLLMMSFAGAAYAHNPVTDEEVYHSFNSHDWQNWNMSDGWKNDDYFFGCHWSQNRVNFYGGQMELSLRTNYSYAPPYNYECAEYTTNNFYGYGLYEVSMKPAKVSGVISSFFTYTGPSYNGAPWDEIDIEFLGNDTTKVQFNYYTDGVGGNEILYDLGFDAADSYNTYAFDWQENYINWYVNGQLVATATENIPSNPSKIMMNIWNTYGIDEWAGRYYGEDANASYNWVRYTPNR

SEQ ID NO: 2 - protein, 379 aa, Bacillus sp
MVKIKINNSIRIVMLTLIMMSVSVVAYAYNPVTEDELYHSFDSHDARNWQISDGWRNGDDFFGCHWSQNRVNFNRGEMELSLRTNYSYSAPYNYECAEYATSNFYGYGLYEVSMKPANVSGVISSFFTYTGPSYNGAPWDEIDIEFLGNDTTKVQFNYYTNGVGGNEIIYDLGFDAANSFNTYAFDWQENYISWYVNGNLVATATENIPSNPSKIMMNVWNTYGIDEWAGAYGGEAANATYEWVRYTPNNGNTTPSTAPDFQLQACDYSDSSGITSWSCGVGTFHSSNWIKFDSVDLSTGYNAFAVSYTSPGSGSFDIRLGSPHGQRIGTVNYGATGGWSNYEWSGTPSLDVTVRGAHDIYIVATSGAANLREFWFKNE

SEQ ID NO: 3 - protein, 276 aa, Bacillus akibai
MKKKFVLFSMCLLLFSGLITGLVQSPQVAEAAERPIGTTFVETFESYDSERWSKAGVWTNGQMFNATWYPEQVTFSDGKMKLQIDKEDNETASPPYKAGELRTNDFYHYGLFEVSMKPAKSTGTVSSFFTYTGPWDWDNDPWDEIDIEFLGKDTTKIQFNYFTNGVGGNEHYHELGFDAADDFNTYAFEWRPESIRWFVNGELVHTATENIPQTPQKIMMNLWPGIGVDGWTGRFNGEDTPVVTQYDWVKYTPLEELGCYNEKNNKYKKCKKTKVK

SEQ ID NO: 4 - protein, 243 aa, Bacillus mojavensis
MSYRMKRVLLLLVTGLFMSLSAFTSTASAQTGGSFFDPFNGYNSGFWQKANGYSNGNMFNCTWRANNVSMTSLGEMRLALTSPSYNKFDCGENRSVQTYGYGLYEVRMKPAKNVGIVSSFFTYTGPTDGTPWDEIDIEFLGKDTTKVQFNYYTNGVGNHEKLVDLGFDAANAYHTYAFDWQPNSIKWYVDGQLKHTATSQIPTTPGKIMMNLWNGTGVDEWLGSYNGVTPLYAHYDWVRYTKK

SEQ ID NO: 5 - protein, 214 aa, Bacillus amyloliquefaciens
QTGGSFFEPFNSYNSGLWQKANGYSNGDMFNCTWRANNVSMTSSGEMRLALTSPSYNKFDCGENRSVQTYGYGLYEVRMKPAKNTGIVSSFFTYTGPTDGTPWDEIDIEFLGKDTTKVQFNYYTNGAGNHEKVADLGFDATNAYHTYAFDWQPNSIKWYVDGQLKHTATSQIPTNPGKIMMNLWNGIGVDDWLGSYNGVNPLYAHYDWVRYTKK

SEQ ID NO: 6 - protein, 214 aa, Bacillus subtilis
QTGGSFFDPFNGYNSGFWQKADGYSNGNMFNCTWRANNVSMTSLGEMRLALTSPAYNKFDCGENRSVQTYGYGLYEVRMKPAKNTGIVSSFFTYTGPTDGTPWDEIDIEFLGKDTTKVQFNYYTNGAGNHEKIVDLGFDAANAYHTYAFDWQPNSIKWYVDGQLKHTATNQIPTTPGKIMMNLWNGTGVDEWLGSYNGVNPLYAHYDWVRYTKK